European Patent Application EP 4 644 361 A1, published November 5, 2025. Title: Lipid nanoparticle formulation comprising of ionizable lipid having branched structure and their use of. Applicant: 이화여자대학교 산학협력단. The sequence listing filed with the application follows.

SEQUENCE LISTING (5 sequences)

SEQ ID NO: 1 - RNA, 1653 nt, unidentified
  source 1..1653: mol_type = mRNA
atggaagacgccaaaaacataaagaaaggcccggcgccattctatccgctggaagatggaaccgctggagagcaactgcataaggctatgaagagatacgccctggttcctggaacaattgcttttacagatgcacatatcgaggtggacatcacttacgctgagtacttcgaaatgtccgttcggttggcagaagctatgaaacgatatgggctgaatacaaatcacagaatcgtcgtatgcagtgaaaactctcttcaattctttatgccggtgttgggcgcgttatttatcggagttgcagttgcgcccgcgaacgacatttataatgaacgtgaattgctcaacagtatgggcatttcgcagcctaccgtggtgttcgtttccaaaaaggggttgcaaaaaattttgaacgtgcaaaaaaagctcccaatcatccaaaaaattattatcatggattctaaaacggattaccagggatttcagtcgatgtacacgttcgtcacatctcatctacctcccggttttaatgaatacgattttgtgccagagtccttcgatagggacaagacaattgcactgatcatgaactcctctggatctactggtctgcctaaaggtgtcgctctgcctcatagaactgcctgcgtgagattctcgcatgccagagatcctatttttggcaatcaaatcattccggatactgcgattttaagtgttgttccattccatcacggttttggaatgtttactacactcggatatttgatatgtggatttcgagtcgtcttaatgtatagatttgaagaagagctgtttctgaggagccttcaggattacaagattcaaagtgcgctgctggtgccaaccctattctccttcttcgccaaaagcactctgattgacaaatacgatttatctaatttacacgaaattgcttctggtggcgctcccctctctaaggaagtcggggaagcggttgccaagaggttccatctgccaggtatcaggcaaggatatgggctcactgagactacatcagctattctgattacacccgagggggatgataaaccgggcgcggtcggtaaagttgttccattttttgaagcgaaggttgtggatctggataccgggaaaacgctgggcgttaatcaaagaggcgaactgtgtgtgagaggtcctatgattatgtccggttatgtaaacaatccggaagcgaccaacgccttgattgacaaggatggatggctacattctggagacatagcttactgggacgaagacgaacacttcttcatcgttgaccgcctgaagtctctgattaagtacaaaggctatcaggtggctcccgctgaattggaatccatcttgctccaacaccccaacatcttcgacgcaggtgtcgcaggtcttcccgacgatgacgccggtgaacttcccgccgccgttgttgttttggagcacggaaagacgatgacggaaaaagagatcgtggattacgtcgccagtcaagtaacaaccgcgaaaaagttgcgcggaggagttgtgtttgtggacgaagtaccgaaaggtcttaccggaaaactcgacgcaagaaaaatcagagagatcctcataaaggccaagaagggcggaaagatcgccgtgtaa

SEQ ID NO: 2 - RNA, 582 nt, Homo sapiens
  source 1..582: mol_type = mRNA
atgggcgtgcacgagtgccccgcctggctgtggctgctgctgagcctgctgagcctgcccctgggcctgcccgtgctgggcgcccccccccggctgatctgcgacagccgggtgctggagcggtacctgctggaggccaaggaggccgagaacatcaccaccggctgcgccgagcactgcagcctgaacgagaacatcaccgtgcccgacaccaaggtgaacttctacgcctggaagcggatggaggtgggccagcaggccgtggaggtgtggcagggcctggccctgctgagcgaggccgtgctgcggggccaggccctgctggtgaacagcagccagccctgggagcccctgcagctgcacgtggacaaggccgtgagcggcctgcggagcctgaccaccctgctgcgggccctgggcgcccagaaggaggccatcagcccccccgacgccgccagcgccgcccccctgcggaccatcaccgccgacaccttccggaagctgttccgggtgtacagcaacttcctgcggggcaagctgaagctgtacaccggcgaggcctgccggaccggcgaccggtga

SEQ ID NO: 3 - RNA, 3828 nt, unidentified
  source 1..3828: mol_type = mRNA
atgttcgtgttcctggtgctgctgcccctggtgagcagccagtgcgtgaacctgaccacccggacccagctgccaccagcctacaccaacagcttcacccggggcgtctactaccccgacaaggtgttccggagcagcgtcctgcacagcacccaggacctgttcctgcccttcttcagcaacgtgacctggttccacgccatccacgtgagcggcaccaacggcaccaagcggttcgacaaccccgtgctgcccttcaacgacggcgtgtacttcgccagcaccgagaagagcaacatcatccggggctggatcttcggcaccaccctggacagcaagacccagagcctgctgatcgtgaataacgccaccaacgtggtgatcaaggtgtgcgagttccagttctgcaacgaccccttcctgggcgtgtactaccacaagaacaacaagagctggatggagagcgagttccgggtgtacagcagcgccaacaactgcaccttcgagtacgtgagccagcccttcctgatggacctggagggcaagcagggcaacttcaagaacctgcgggagttcgtgttcaagaacatcgacggctacttcaagatctacagcaagcacaccccaatcaacctggtgcgggatctgccccagggcttctcagccctggagcccctggtggacctgcccatcggcatcaacatcacccggttccagaccctgctggccctgcaccggagctacctgaccccaggcgacagcagcagcgggtggacagcaggcgcggctgcttactacgtgggctacctgcagccccggaccttcctgctgaagtacaacgagaacggcaccatcaccgacgccgtggactgcgccctggaccctctgagcgagaccaagtgcaccctgaagagcttcaccgtggagaagggcatctaccagaccagcaacttccgggtgcagcccaccgagagcatcgtgcggttccccaacatcaccaacctgtgccccttcggcgaggtgttcaacgccacccggttcgccagcgtgtacgcctggaaccggaagcggatcagcaactgcgtggccgactacagcgtgctgtacaacagcgccagcttcagcaccttcaagtgctacggcgtgagccccaccaagctgaacgacctgtgcttcaccaacgtgtacgccgacagcttcgtgatccgtggcgacgaggtgcggcagatcgcacccggccagacaggcaagatcgccgactacaactacaagctgcccgacgacttcaccggctgcgtgatcgcctggaacagcaacaacctcgacagcaaggtgggcggcaactacaactacctgtaccggctgttccggaagagcaacctgaagcccttcgagcgggacatcagcaccgagatctaccaagccggctccaccccttgcaacggcgtggagggcttcaactgctacttccctctgcagagctacggcttccagcccaccaacggcgtgggctaccagccctaccgggtggtggtgctgagcttcgagctgctgcacgccccagccaccgtgtgtggccccaagaagagcaccaacctggtgaagaacaagtgcgtgaacttcaacttcaacggccttaccggcaccggcgtgctgaccgagagcaacaagaaattcctgccctttcagcagttcggccgggacatcgccgacaccaccgacgctgtgcgggatccccagaccctggagatcctggacatcaccccttgcagcttcggcggcgtgagcgtgatcaccccaggcaccaacaccagcaaccaggtggccgtgctgtaccaggacgtgaactgcaccgaggtgcccgtggccatccacgccgaccagctgacacccacctggcgggtctacagcaccggcagcaacgtgttccagacccgggccggttgcctgatcggcgccgagcacgtgaacaacagctacgagtgcgacatccccatcggcgccggcatctgtgccagctaccagacccagaccaattcaccccggagggcaaggagcgtggccagccagagcatcatcgcctacaccatgagcctgggcgccgagaacagcgtggcctacagcaacaacagcatcgccatccccaccaacttcaccatcagcgtgaccaccgagattctgcccgtgagcatgaccaagaccagcgtggactgcaccatgtacatctgcggcgacagcaccgagtgcagcaacctgctgctgcagtacggcagcttctgcacccagctgaaccgggccctgaccggcatcgccgtggagcaggacaagaacacccaggaggtgttcgcccaggtgaagcagatctacaagacccctcccatcaaggacttcggcggcttcaacttcagccagatcctgcccgaccccagcaagcccagcaagcggagcttcatcgaggacctgctgttcaacaaggtgaccctagccgacgccggcttcatcaagcagtacggcgactgcctcggcgacatagccgcccgggacctgatctgcgcccagaagttcaacggcctgaccgtgctgcctcccctgctgaccgacgagatgatcgcccagtacaccagcgccctgttagccggaaccatcaccagcggctggactttcggcgctggagccgctctgcagatccccttcgccatgcagatggcctaccggttcaacggcatcggcgtgacccagaacgtgctgtacgagaaccagaagctgatcgccaaccagttcaacagcgccatcggcaagatccaggacagcctgagcagcaccgctagcgccctgggcaagctgcaggacgtggtgaaccagaacgcccaggccctgaacaccctggtgaagcagctgagcagcaacttcggcgccatcagcagcgtgctgaacgacatcctgagccggctggaccctcccgaggccgaggtgcagatcgaccggctgatcactggccggctgcagagcctgcagacctacgtgacccagcagctgatccgggccgccgagattcgggccagcgccaacctggccgccaccaagatgagcgagtgcgtgctgggccagagcaagcgggtggacttctgcggcaagggctaccacctgatgagctttccccagagcgcaccccacggagtggtgttcctgcacgtgacctacgtgcccgcccaggagaagaacttcaccaccgccccagccatctgccacgacggcaaggcccactttccccgggagggcgtgttcgtgagcaacggcacccactggttcgtgacccagcggaacttctacgagccccagatcatcaccaccgacaacaccttcgtgagcggcaactgcgacgtggtgatcggcatcgtgaacaacaccgtgtacgatcccctgcagcccgagctggacagcttcaaggaggagctggacaagtacttcaagaatcacaccagccccgacgtggacctgggcgacatcagcggcatcaacgccagcgtggtgaacatccagaaggagatcgatcggctgaacgaggtggccaagaacctgaacgagagcctgatcgacctgcaggagctgggcaagtacgagcagtacatcaagtggccctggtacatctggctgggcttcatcgccggcctgatcgccatcgtgatggtgaccatcatgctgtgctgcatgaccagctgctgcagctgcctgaagggctgttgcagctgcggcagctgctgcaagttcgacgaggacgacagcgagcccgtgctgaagggcgtgaagctgcactacacctgataatag

SEQ ID NO: 4 - RNA, 3801 nt, unidentified
  source 1..3801: mol_type = mRNA
atgttcgtgtttctggtcctgctgcctctggtgtctagccagtgcgtgaacctgaccacccggacccaactgcctcctgcctacaccaatagctttacaagaggcgtgtattaccccgataaggtgttcagaagcagcgtgctgcacagcacaaccgacctgttcctgcctttcttcagcaacgtgacctggttccacgccatcagcggaactaacggcaccaagagattcgacaaccccgtgctgccattcaacgacggcgtttatttcgcctctaccgagaagagcaacatcatcagaggctggatcttcggcaccaccctggacagcaaaacccagagtctgctgatcgtgaataacgccaccaacgtcgtcatcaaggtgtgcgagttccagttctgcaacgaccctttcttgggcgtgtaccacaagaacaacaagtcctggatggaaagcgaatttagagtgtacgactctgccaacaactgcaccttcgagtacgtgtccagccctttcctgatggaccttgaaggaaaacagggcaacttcaagaatctgagggaattcgtgttcaaaaacatcgacggctacttcaagatctacagcaagcacacccctatcaacctggtgcgggacttgccgcaaggcttcagcgccctggaacctctggtggacctgcccatcggcattaacatcacccggttccagaccctgctggccctccacagatcctacctgacccctggcgatagctctcagggctggaccgccggcgccgctgcttactacgtgggatacctgcagcctagaacattcctgctgaagtacaacgagaacggcacaatcaccgacgccgtggactgcgccctggaccccctgtctgagacaaagtgcacactgaaaagcttcaccgtggaaaaaggcatctaccaaaccagcaatttcagagtgcagcctacagattccatcgtgcggtttccaaatatcacaaacctgtgtccttttggcgaggtgttcaacgccaccagattcgcctccgtgtatgcctggaacagaaagagaatcagcaactgcgtggccgactacagcgtgctgtacaacagcgcctcctttagcacattcaagtgctacggcgtcagccctacaaagctgaacgacctgtgcttcaccaacgtctacgccgacagctttgtgatccggggcgacgaggtgcggcagatcgcccctggccagactggcaagatcgctgactacaattataagctgccagatgacttcaccggatgtgtgatcgcctggaactccaacaacctggatagcaaggtgggcggaaattacaactacagataccggctgttccggaagtctaacctgaagccttttgaaagagatattagcactgagatctaccaggccggcagcaagccctgtaatggagtggaaggcttcaactgctactttcctctgcaaagctacgggtttcagcctacaaatggcgtgggctaccagccctacagagtggtggtgctgagcttcgagctgctgcatgctcctgctacagtgtgcggccctaagaagtccacaaatctggtgaagaacaaatgtgtgaacttcaatttcaacggcctgacaggcaccggcgttctgacagagagcaacaagaaattcctgcccttccagcagttcggcagagacatcgcagatacaaccgatgccgtgagagatccccagaccctggagatcctggacatcaccccctgtagcttcggcggcgttagcgtgatcaccccaggcaccaatacctctaaccaggtcgctgtgctgtaccagggagtgaactgcaccgaggtgcctgtggctatccacgccgatcagctgacccccacatggcgggtgtactctacaggaagcaatgtgtttcagacccgcgccggttgtctgatcggcgccgagcacgtgaacaattcatacgagtgcgacatccctatcggagctggcatctgcgcctcctaccagacccagaccaacagccccgcctctgtagcctctcaaagcatcattgcctacacaatgagcctgggcgccgagaactccgttgcttatagtaataatagcattgcaatccctaccaacttcaccatcagcgtgaccacagagattctgcctgtgagcatgaccaagacctccgtggactgtaccatgtacatctgtggcgactcgactgaatgcagcaacctgctgctccaatacggcagcttctgcacacagctgaaccgggctctgaccggcatcgccgtggaacaggacaagaacacccaagaggtgtttgcccaggtgaagcagatttacaagacccctcccatcaaggacttcggcggtttcaactttagccagatcctgcctgatccttctaaacccagcaagcggagccccatcgaggacctgctgttcaacaaggtgaccctggctgacgccggattcatcaagcagtatggcgactgtctgggcgatatcgctgccagagacctcatctgtgcccagaagttcaacggactgactgtgctaccacccttactgaccgatgagatgatcgctcagtacacatctgccctgctggctgggaccatcaccagcggctggacattcggcgccggccccgccctgcaaatcccgtttcctatgcagatggcctatagattcaacggaatcggcgtgacccagaacgtcctgtatgagaaccagaagctgatcgctaatcagttcaacagcgcaatcggcaaaatccaagactctctgagcagcacaccctccgctctgggcaagctgcaggatgtggtgaaccaaaacgcccaagcccttaacaccctggtgaaacagctgagcagcaactttggtgccatcagcagcgtgcttaacgacattctgtctaggctggacccccctgaggccgaagtgcagatcgacagactgatcaccggaagactgcagagcctgcaaacctacgtgacccaacagttgatcagagccgctgagatccgggcgagcgccaacctggccgccacaaagatgagcgaatgtgtgctggggcagagcaaaagagtggacttctgcggcaaaggctatcacctgatgagctttcctcagagcgccccccacggcgtggtgttcctgcacgtgacatacgtgcctgctcaggagaagaacttcaccaccgcccctgccatctgccacgacggcaaggctcacttcccaagagaaggcgtgttcgtcagcaatggcacccactggttcgtgacccaaagaaacttctacgagcctcagatcatcacaaccgacaacacattcgtgagcgggaactgcgacgtggtaatcggcattgtgaacaataccgtgtacgaccctctgcagccagaactggattccttcaaggaagagctggacaagtactttaagaaccacacaagccctgacgtggacctgggcgacataagcggtatcaacgcctcagtggtcaacatccagaaagagatcgacaggttaaacgaagtggccaagaacctgaatgagtccctgatcgatctgcaggagctgggcaagtacgaacagtacatcaagtggccttggtacatctggctgggattcattgccggattgatcgccatcgtcatggtgaccatcatgctgtgctgcatgacgagctgctgctcttgcctgaagggctgctgtagctgtggctcctgttgtaaattcgacgaagatgacagcgagcccgtgctgaagggagtgaagctgcattacacc

SEQ ID NO: 5 - RNA, 378 nt, unidentified
  source 1..378: mol_type = mRNA
atggacgccatgaagcggggcctgtgctgcgtgctgctcctgtgcggcgctgtgtttgtgagccctagcgtgaagaccaaaaacaccaccactacacaaacccagccgagcaagcccaccaccaaacagcgccagaataagcccccatccaagcccaacaacgacttccacttcgaggtattcaatttcgtgccctgttccatctgttcaaacaatcccacctgctgggccatctgcaagcggattcccaataagaagcccggcaagaagaccacgaccaagcccacgaagaagcctacgctgaagaccaccaaaaaagaccctaagccccagaccacgaagtccaaggaggtgcccaccaccaagcctctcgagtaa